European Patent Application EP 4 530 350 A2, published April 2, 2025. Title: IMPROVED FLARE (FLOW CYTOMETRY ATTENUATED REPORTER EXPRESSION) TECHNOLOGY FOR RAPID BULK SORTING. Applicant: Genzyme Corporation. Application EP Divisional of EP16788602.7, filed November 12, 2024. The sequence listing filed with the application follows.

SEQUENCE LISTING (8 sequences)

SEQ ID NO: 1 - protein, 61 aa, Homo sapiens
LERFLFLLLTISLLVLVQIQTGLSGQNDTSQTSSPSASSNISGGIFLFFVANAIIHLFCFS

SEQ ID NO: 2 - protein, 128 aa, Homo sapiens
LGIQGGSVLFGLLLVLAVFCHSGHSLQCYNCPNPTADCKTAVNCSSDFDACLITKAGLQVYNNCWKFEHCNFNDVTTRLRENELTYYCCKKDLCNFNEQLENGGTSLSEKTVLLLVTPFLAAAWSLHP

SEQ ID NO: 3 - protein, 74 aa, Mus sp.
LKSFLLFLTIILLVVIQIQTGSLGQATTAASGTNKNSTSTKKTPLKSGASSIIDAGACSFLFFANTLICLFYLS

SEQ ID NO: 4 - DNA, 186 bp, Homo sapiens
  source 1..186: mol_type = other DNA
ttggagcgcttcctcttcctcctactcaccatcagcctcctcgttttggtacaaatacaaaccggactctccggacaaaacgacaccagccaaaccagcagcccctcagcatccagcaacataagcggaggcattttccttttcttcgtcgccaacgccataatccacctcttctgcttcagttga

SEQ ID NO: 5 - DNA, 387 bp, Homo sapiens
  source 1..387: mol_type = other DNA
ttgggaatccaaggagggtctgtcctgttcgggctgctgctcgtcctcgctgtcttctgccattccggtcatagcctgcagtgctacaactgtcctaacccaactgctgactgcaaaacagccgtcaattgttcatctgattttgacgcgtgtctcattaccaaagctgggttacaagtgtataacaactgttggaagtttgagcattgcaatttcaacgacgtcacaacccgcttgagggaaaacgagctaacgtactactgctgcaagaaggacctgtgtaactttaacgaacagcttgaaaacggagggacatccttatcagagaaaacagttcttctgctggtgactccatttctggcagctgcttggagccttcatccctaa

SEQ ID NO: 6 - DNA, 233 bp, Mus sp.
  source 1..233: mol_type = other DNA
ttgaagagcttcctcctcttcctcactatcattcttctcgtagtcattcagatacaaacaggatccttaggacaagccactacggccgcttcaggtactaacaaaaacagcacctccaccaaaaaaacccccttaaagagcggggcctcatccatcatcgacgcgggcgcttgcagtttcctcttcttcgccaatacccttatttgcctcttctacctcagctaactgagtaa

SEQ ID NO: 7 - DNA, 8123 bp, synthetic construct
  misc_feature 1..8123: note = source = /note="Description of Artificial Sequence: Synthetic polynucleotide"
  source 1..8123: mol_type = other DNA
ggatccgctgtggaatgtgtgtcagttagggtgtggaaagtccccaggctccccagcaggcagaagtatgcaaagcatgcatctcaattagtcagcaaccaggtgtggaaagtccccaggctccccagcaggcagaagtatgcaaagcatgcatctcaattagtcagcaaccatagtcccgcccctaactccgcccatcccgcccctaactccgcccagttccgcccattctccgccccatggctgactaattttttttatttatgcagaggccgaggccgcctcggcctctgagctattccagaagtagtgaggaggcttttttggaggcctaggcttttgcaaaaagcttggggggggggacagctcagggctgcgatttcgcgccaaacttgacggcaatcctagcgtgaaggctggtaggattttatccccgctgccatcatggttcgaccattgaactgcatcgtcgccgtgtcccaaaatatggggattggcaagaacggagacctaccctggcctccgctcaggaacgagttcaagtacttccaaagaatgaccacaacctcttcagtggaaggtaaacagaatctggtgattatgggtaggaaaacctggttctccattcctgagaagaatcgacctttaaaggacagaattaatatagttctcagtagagaactcaaagaaccaccacgaggagctcattttcttgccaaaagtttggatgatgccttaagacttattgaacaaccggaattggcaagtaaagtagacatggtttggatagtcggaggcagttctgtttaccaggaagccatgaatcaaccaggccacctcagactctttgtgacaaggatcatgcaggaatttgaaagtgacacgtttttcccagaaattgatttggggaaatataaacttctcccagaatacccaggcgtcctctctgaggtccaggaggaaaaaggcatcaagtataagtttgaagtctacgagaagaaagactaacaggaagatgctttcaagttctctgctcccctcctaaagctatgcatttttataagaccatgggacttttgctggctttagatctttgtgaaggaaccttacttctgtggtgtgacataattggacaaactacctacagagatttaaagctctaaggtaaatataaaatttttaagtgtataatgtgttaaactactgattctaattgtttgtgtattttagattccaacctatggaactgatgaatgggagcagtggtggaatgcctttaatgaggaaaacctgttttgctcagaagaaatgccatctagtgatgatgaggctactgctgactctcaacattctactcctccaaaaaagaagagaaaggtagaagaccccaaggactttccttcagaattgctaagttttttgagtcatgctgtgtttagtaatagaactcttgcttgctttgctatttacaccacaaaggaaaaagctgcactgctatacaagaaaattatggaaaaatattctgtaacctttataagtaggcataacagttataatcataacatactgttttttcttactccacacaggcatagagtgtctgctattaataactatgctcaaaaattgtgtacctttagctttttaatttgtaaaggggttaataaggaatatttgatgtatagtgccttgactagagatcataatcagccataccacatttgtagaggttttacttgctttaaaaaacctcccacacctccccctgaacctgaaacataaaatgaatgcaattgttgttgttaacttgtttattgcagcttataatggttacaaataaagcaatagcatcacaaatttcacaaataaagcatttttttcactgcattctagttgtggtttgtccaaactcatcaatgtatcttatcatgtctggatcctctacgccggacgcatcgtggccggcatcaccggcgccacaggtgcggttgctggcgcctatatcgccgacatcaccgatggggaagatcgggctcgccacttcgggctcatgagcgcttgtttcggcgtgggtatggtggcaggccgtggccgggggactgttgggcgccatctccttgcatgcaccattccttgcggcggcggtgctcaacggcctcaacctactactgggctgcttcctaatgcaggagtcgcataagggagagcgtcgaccgatgcccttgagagccttcaacccagtcagctccttccggtgggcgcggggcatgactatcgtcgccgcacttatgactgtcttctttatcatgcaactcgtaggacaggtgccggcagcgctctgggtcattttcggcgaggaccgctttcgctggagcgcgacgatgatcggcctgtcgcttgcggtattcggaatcttgcacgccctcgctcaagccttcgtcactggtcccgccaccaaacgtttcggcgagaagcaggccattatcgccggcatggcggccgacgcgctgggctacgtcttgctggcgttcgcgacgcgaggctggatggccttccccattatgattcttctcgcttccggcggcatcgggatgcccgcgttgcaggccatgctgtccaggcaggtagatgacgaccatcagggacagcttcaaggccagcaaaaggccaggaaccgtaaaaaggccgcgttgctggcgtttttccataggctccgcccccctgacgagcatcacaaaaatcgacgctcaagtcagaggtggcgaaacccgacaggactataaagataccaggcgtttccccctggaagctccctcgtgcgctctcctgttccgaccctgccgcttaccggatacctgtccgcctttctcccttcgggaagcgtggcgctttctcatagctcacgctgtaggtatctcagttcggtgtaggtcgttcgctccaagctgggctgtgtgcacgaaccccccgttcagcccgaccgctgcgccttatccggtaactatcgtcttgagtccaacccggtaagacacgacttatcgccactggcagcagccactggtaacaggattagcagagcgaggtatgtaggcggtgctacagagttcttgaagtggtggcctaactacggctacactagaaggacagtatttggtatctgcgctctgctgaagccagttaccttcggaaaaagagttggtagctcttgatccggcaaacaaaccaccgctggtagcggtggtttttttgtttgcaagcagcagattacgcgcagaaaaaaaggatctcaagaagatcctttgatcttttctacggggtctgacgctcagtggaacgaaaactcacgttaagggattttggtcatgagattatcaaaaaggatcttcacctagatccttttaaattaaaaatgaagttttaaatcaatctaaagtatatatgagtaaacttggtctgacagttaccaatgcttaatcagtgaggcacctatctcagcgatctgtctatttcgttcatccatagttgcctgactccccgtcgtgtagataactacgatacgggagggcttaccatctggccccagtgctgcaatgataccgcgagacccacgctcaccggctccagatttatcagcaataaaccagccagccggaagggccgagcgcagaagtggtcctgcaactttatccgcctccatccagtctattaattgttgccgggaagctagagtaagtagttcgccagttaatagtttgcgcaacgttgttgccattgctgcaggcatcgtggtgtcacgctcgtcgtttggtatggcttcattcagctccggttcccaacgatcaaggcgagttacatgatcccccatgttgtgcaaaaaagcggttagctccttcggtcctccgatcgttgtcagaagtaagttggccgcagtgttatcactcatggttatggcagcactgcataattctcttactgtcatgccatccgtaagatgcttttctgtgactggtgagtactcaaccaagtcattctgagaatagtgtatgcggcgaccgagttgctcttgcccggcgtcaacacgggataataccgcgccacatagcagaactttaaaagtgctcatcattggaaaacgttcttcggggcgaaaactctcaaggatcttaccgctgttgagatccagttcgatgtaacccactcgtgcacccaactgatcttcagcatcttttactttcaccagcgtttctgggtgagcaaaaacaggaaggcaaaatgccgcaaaaaagggaataagggcgacacggaaatgttgaatactcatactcttcctttttcaatattattgaagcatttatcagggttattgtctcatgagcggatacatatttgaatgtatttagaaaaataaacaaataggggttccgcgcacatttccccgaaaagtgccacctgacgtctaagaaaccattattatcatgacattaacctataaaaataggcgtatcacgaggccctttcgtcttcaagaattggggaccaagacagaaccataagccagtgggatagatcagaaatgttccagaggtgggatggggccagagtgcctgccccttgaaccgtcccagggaccagaggtgacaaagtggcaacacaggtcctgcctgggaatctggtctgctcctacttagtaaagctgcctggtgtcacacaagaggcccccacttattcctgcacccctggtggtaggtggcgtcttctcccctgcagccaccaggctcccctgagaacactgccggcagtcctcattgacaggcagtattcgctctgccccacccccacctgtgaattgcagggctggcaggtcctcaggcagctggcaaaccgcctgaacaactgagagatacagggccagggccagggcagtcccgtcccccggaggcagggaggggacgtgctgggaaagttctctctctcaggcccaggttggtgactgcagaaggcttctgtcaaatctcttttgtgggaaccacagagtagccctgaacgtgggggtgtgcttccagtatactctggggtcaccctttccatactggaggcctctgcaacttcaaaatgctctgctaccaacctagcacaaggaagttggtccagcctccccacgcagggccactgctgcagtccatatatggactaagccttccttggtttcaacacctacactcactgagcccctactatgtgtatgcagagccgagacaggccctgagcatctcatctgaagcacccttcttgcctaaattcagttttctgtcactttctcccaggaggtgtgtgtccctctaagctaagccaggggtccctcacccctgccccactcccatccctagtgtaggtatcagctgaagagcttcctgagcagaacactcttgggtgctgacattttgataaataggcccatgtttaggagagcaggggtccgggggcgggagatcttctctggtggattgagggctccaagaactactctttgagcacgctgcccctcccagagtccccacagcctccagatggactagaacacagttcggctgtggctgcacataactaacagaggatagatggtgggtcccagcccaacagtgcctggcaatcacccagagccaccagctaacggccttggcttagttttttgcctgggtgtgatcaggcagccctccaaaactgcccggactccatgacaagttttgcttgttctatagagcacagttcctttctaggtctggggcaagggacatcgggagacatcttcctgcaacagctccagtcactggaccaccaggctcgccctgtctttggtgtgtggccctgagtctcctaagtggcccaaacctgtgaagacccctccaaccacagttttgcttctaaattgtaccccaacacacctagcaaattgaaaccccaccagaagtcccccagatctggctttccggctattgctggcaagggggagtgactcccggcccattcaatccaggccccgcgtgttcctcaaacaagaagccacgtaaacataaaccgagcctccatgctgacccttgcccatcgaggtactcaatgttcacgtgatatccacacccagagggtcctggggtgggtgcatgagccccagaatgcaggcttgataaccgagaccctgaatcgggcagtgtccacaagggcggaggccagtcatgcatgttcgggcctatggggccagcacccaacgccaaaactctccatcctcttcctcaatctcgctttctctctctctctctttttttttttttattttttttttttgcaaaaggaggggagagggggtaaaaaaatgctgcactgtgcggctaggccggtgagtgagcggcgcggagccaatcagcgctcgccgttccgaaagttgccttttatggctcgagtggccgctgtggcgtcctataaaacccggcggcgcaacgcgcagccactgtcgagtccgcgtccacccgcgagcacaggcctttcgcagctctttcttcgccgctccacacccgccaccaggtaagcagggacaacaggcccagccggccacagccctcccgtgggcagtgaccgcgctgcagggtcgcgggggacactcggcgcggacaccggggaaggctggagggtggtgccgggccgcggagcggacactttcagatccaactttcagtccagggtgtagaccctttacagccgcattgccacggtgtagacaccggtggacccgctctggctcagagcacgcggcttgggggaacccattagggtcgcagtgtgggcgctatgagagccgatgcagctttcgggtgttgaaccgtatctgcccaccttggggggaggacacaaggtcgggagccaaacgccacgatcatgccttggtggcccatgggtctttgtctaaaccggtttgcccatttggcttgccgggcgggcgggcgcggcgggcccggctcggccgggtgggggctgggttgccactgcgcttgcgcgctctatggctgggtattggggcgcgtgcacgctggggagggagcccttcctcttccccctctcccaagttaaacttgcgcgtgcgtattgagacttggagcgcggccaccggggttgggcgagggcggggccgttgtccggaaggggcggggtcgcagcggcttcggggcgcctgctcgcgcttcctgctgggtgtggtcgcctcccgcgcgcgcactagccgcccgccggcggggcgaaggcggggcttgcgcccgtttggggagggggcggaggcctggcttcctgccgtggggccgcctccggaccagcgtttgcctcttatggtaataacgcggccggcctgggcttcctttgtcccctgagtttgggcgcgcgccccctggcggcccgaggccgcggcttgccggaagtgggcagggcggcagcggctgcgcctagtggcccgctagtgaccgcgaccctcttttgtgccctgatatagttcgccggatcctaccgcggtagcggccgcgccaccttggagcgcttcctcttcctcctactcaccatcagcctcctcgttttggtacaaatacaaaccggactctccggacaaaacgacaccagccaaaccagcagcccctcagcatccagcaacataagcggaggcattttccttttcttcgtcgccaacgccataatccacctcttctgcttcagttgaaggccggccaatacgtaggcgcgccattgagtgagtgatttggcgcgccaagatatcacacccgggattaattaaaggtacctacgcgtagaattccacgtagtggtttaaactctagatactcgagggatctggatcataatcagccataccacatttgtagaggttttacttgctttaaaaaacctcccacacctccccctgaacctgaaacataaaatgaatgcaattgttgttgttaacttgtttattgcagcttataatggttacaaataaagcaatagcatcacaaatttcacaaataaagcatttttttcactgcattctagttgtggtttgtccaaactcatcaatgtatcttatcatgtct

SEQ ID NO: 8 - DNA, 10 bp, synthetic construct
  misc_feature 1..10: note = source = /note="Description of Artificial Sequence: Synthetic oligonucleotide"
  source 1..10: mol_type = other DNA
gccrccatgg